European Patent Specification EP 3 955 960 B1, published January 15, 2025. Title: IPILIMUMAB VARIANTS WITH ENHANCED SPECIFICITY FOR BINDING AT LOW PH. Applicant: Bristol-Myers Squibb Company. The sequence listing filed with the application follows.

SEQUENCE LISTING (44 sequences)

SEQ ID NO: 1 - protein, 223 aa, Homo sapiens
MACLGFQRHKAQLNLATRTWPCTLLFFLLFIPVFCKAMHVAQPAVVLASSRGIASFVCEYASPGKATEVRVTVLRQADSQVTEVCAATYMMGNELTFLDDSICTGTSSGNQVNLTIQGLRAMDTGLYICKVELMYPPPYYLGIGNGTQIYVIDPEPCPDSDFLLWILAAVSSGLFFYSFLLTAVSLSKMLKKRSPLTTGVYVKMPPTEPECEKQFQPYFIPIN

SEQ ID NO: 2 - protein, 220 aa, Homo sapiens
MLRLLLALNLFPSIQVTGNKILVKQSPMLVAYDNAVNLSCKYSYNLFSREFRASLHKGLDSAVEVCVVYGNYSQQLQVYSKTGFNCDGKLGNESVTFYLQNLYVNQTDIYFCKIEVMYPPPYLDNEKSNGTIIHVKGKHLCPSPLFPGPSKPFWVLVVVGGVLACYSLLVTVAFIIFWVRSKRSRLLHSDYMNMTPRRPGPTRKHYQPYAPPRDFAAYRS

SEQ ID NO: 3 - protein, 10 aa, Homo sapiens
GFTFSSYTMH

SEQ ID NO: 4 - protein, 17 aa, Homo sapiens
FISYDGNNKYYADSVKG

SEQ ID NO: 5 - protein, 9 aa, Homo sapiens
TGWLGPFDY

SEQ ID NO: 6 - protein, 12 aa, Homo sapiens
RASQSVGSSYLA

SEQ ID NO: 7 - protein, 7 aa, Homo sapiens
GAFSRAT

SEQ ID NO: 8 - protein, 9 aa, Homo sapiens
QQYGSSPWT

SEQ ID NO: 9 - protein, 118 aa, Homo sapiens
QVQLVESGGGVVQPGRSLRLSCAASGFTFSSYTMHWVRQAPGKGLEWVTFISYDGNNKYYADSVKGRFTISRDNSKNTLYLQMNSLRAEDTAIYYCARTGWLGPFDYWGQGTLVTVSS

SEQ ID NO: 10 - protein, 108 aa, Homo sapiens
EIVLTQSPGTLSLSPGERATLSCRASQSVGSSYLAWYQQKPGQAPRLLIYGAFSRATGIPDRFSGSGSGTDFTLTISRLEPEDFAVYYCQQYGSSPWTFGQGTKVEIK

SEQ ID NO: 11 - protein, 447 aa, Homo sapiens
QVQLVESGGGVVQPGRSLRLSCAASGFTFSSYTMHWVRQAPGKGLEWVTFISYDGNNKYYADSVKGRFTISRDNSKNTLYLQMNSLRAEDTAIYYCARTGWLGPFDYWGQGTLVTVSSASTKGPSVFPLAPSSKSTSGGTAALGCLVKDYFPEPVTVSWNSGALTSGVHTFPAVLQSSGLYSLSSVVTVPSSSLGTQTYICNVNHKPSNTKVDKRVEPKSCDKTHTCPPCPAPELLGGPSVFLFPPKPKDTLMISRTPEVTCVVVDVSHEDPEVKFNWYVDGVEVHNAKTKPREEQYNSTYRVVSVLTVLHQDWLNGKEYKCKVSNKALPAPIEKTISKAKGQPREPQVYTLPPSRDELTKNQVSLTCLVKGFYPSDIAVEWESNGQPENNYKTTPPVLDSDGSFFLYSKLTVDKSRWQQGNVFSCSVMHEALHNHYTQKSLSLSPG

SEQ ID NO: 12 - protein, 447 aa, Artificial Sequence
  S31H variant of ipilimumab HC
QVQLVESGGGVVQPGRSLRLSCAASGFTFSHYTMHWVRQAPGKGLEWVTFISYDGNNKYYADSVKGRFTISRDNSKNTLYLQMNSLRAEDTAIYYCARTGWLGPFDYWGQGTLVTVSSASTKGPSVFPLAPSSKSTSGGTAALGCLVKDYFPEPVTVSWNSGALTSGVHTFPAVLQSSGLYSLSSVVTVPSSSLGTQTYICNVNHKPSNTKVDKRVEPKSCDKTHTCPPCPAPELLGGPSVFLFPPKPKDTLMISRTPEVTCVVVDVSHEDPEVKFNWYVDGVEVHNAKTKPREEQYNSTYRVVSVLTVLHQDWLNGKEYKCKVSNKALPAPIEKTISKAKGQPREPQVYTLPPSRDELTKNQVSLTCLVKGFYPSDIAVEWESNGQPENNYKTTPPVLDSDGSFFLYSKLTVDKSRWQQGNVFSCSVMHEALHNHYTQKSLSLSPG

SEQ ID NO: 13 - protein, 447 aa, Artificial Sequence
  S31H / N56H variant of ipilimumab HC
QVQLVESGGGVVQPGRSLRLSCAASGFTFSHYTMHWVRQAPGKGLEWVTFISYDGHNKYYADSVKGRFTISRDNSKNTLYLQMNSLRAEDTAIYYCARTGWLGPFDYWGQGTLVTVSSASTKGPSVFPLAPSSKSTSGGTAALGCLVKDYFPEPVTVSWNSGALTSGVHTFPAVLQSSGLYSLSSVVTVPSSSLGTQTYICNVNHKPSNTKVDKRVEPKSCDKTHTCPPCPAPELLGGPSVFLFPPKPKDTLMISRTPEVTCVVVDVSHEDPEVKFNWYVDGVEVHNAKTKPREEQYNSTYRVVSVLTVLHQDWLNGKEYKCKVSNKALPAPIEKTISKAKGQPREPQVYTLPPSRDELTKNQVSLTCLVKGFYPSDIAVEWESNGQPENNYKTTPPVLDSDGSFFLYSKLTVDKSRWQQGNVFSCSVMHEALHNHYTQKSLSLSPG

SEQ ID NO: 14 - protein, 447 aa, Artificial Sequence
  S31H / N56H / T99H variant of ipilimumab HC
QVQLVESGGGVVQPGRSLRLSCAASGFTFSHYTMHWVRQAPGKGLEWVTFISYDGHNKYYADSVKGRFTISRDNSKNTLYLQMNSLRAEDTAIYYCARHGWLGPFDYWGQGTLVTVSSASTKGPSVFPLAPSSKSTSGGTAALGCLVKDYFPEPVTVSWNSGALTSGVHTFPAVLQSSGLYSLSSVVTVPSSSLGTQTYICNVNHKPSNTKVDKRVEPKSCDKTHTCPPCPAPELLGGPSVFLFPPKPKDTLMISRTPEVTCVVVDVSHEDPEVKFNWYVDGVEVHNAKTKPREEQYNSTYRVVSVLTVLHQDWLNGKEYKCKVSNKALPAPIEKTISKAKGQPREPQVYTLPPSRDELTKNQVSLTCLVKGFYPSDIAVEWESNGQPENNYKTTPPVLDSDGSFFLYSKLTVDKSRWQQGNVFSCSVMHEALHNHYTQKSLSLSPG

SEQ ID NO: 15 - protein, 447 aa, Artificial Sequence
  T33H variant of ipilimumab HC
QVQLVESGGGVVQPGRSLRLSCAASGFTFSSYHMHWVRQAPGKGLEWVTFISYDGNNKYYADSVKGRFTISRDNSKNTLYLQMNSLRAEDTAIYYCARTGWLGPFDYWGQGTLVTVSSASTKGPSVFPLAPSSKSTSGGTAALGCLVKDYFPEPVTVSWNSGALTSGVHTFPAVLQSSGLYSLSSVVTVPSSSLGTQTYICNVNHKPSNTKVDKRVEPKSCDKTHTCPPCPAPELLGGPSVFLFPPKPKDTLMISRTPEVTCVVVDVSHEDPEVKFNWYVDGVEVHNAKTKPREEQYNSTYRVVSVLTVLHQDWLNGKEYKCKVSNKALPAPIEKTISKAKGQPREPQVYTLPPSRDELTKNQVSLTCLVKGFYPSDIAVEWESNGQPENNYKTTPPVLDSDGSFFLYSKLTVDKSRWQQGNVFSCSVMHEALHNHYTQKSLSLSPG

SEQ ID NO: 16 - protein, 447 aa, Artificial Sequence
  N57H variant of ipilimumab HC
QVQLVESGGGVVQPGRSLRLSCAASGFTFSSYTMHWVRQAPGKGLEWVTFISYDGNHKYYADSVKGRFTISRDNSKNTLYLQMNSLRAEDTAIYYCARTGWLGPFDYWGQGTLVTVSSASTKGPSVFPLAPSSKSTSGGTAALGCLVKDYFPEPVTVSWNSGALTSGVHTFPAVLQSSGLYSLSSVVTVPSSSLGTQTYICNVNHKPSNTKVDKRVEPKSCDKTHTCPPCPAPELLGGPSVFLFPPKPKDTLMISRTPEVTCVVVDVSHEDPEVKFNWYVDGVEVHNAKTKPREEQYNSTYRVVSVLTVLHQDWLNGKEYKCKVSNKALPAPIEKTISKAKGQPREPQVYTLPPSRDELTKNQVSLTCLVKGFYPSDIAVEWESNGQPENNYKTTPPVLDSDGSFFLYSKLTVDKSRWQQGNVFSCSVMHEALHNHYTQKSLSLSPG

SEQ ID NO: 17 - protein, 447 aa, Artificial Sequence
  T99H variant of ipilimumab HC
QVQLVESGGGVVQPGRSLRLSCAASGFTFSSYTMHWVRQAPGKGLEWVTFISYDGNNKYYADSVKGRFTISRDNSKNTLYLQMNSLRAEDTAIYYCARHGWLGPFDYWGQGTLVTVSSASTKGPSVFPLAPSSKSTSGGTAALGCLVKDYFPEPVTVSWNSGALTSGVHTFPAVLQSSGLYSLSSVVTVPSSSLGTQTYICNVNHKPSNTKVDKRVEPKSCDKTHTCPPCPAPELLGGPSVFLFPPKPKDTLMISRTPEVTCVVVDVSHEDPEVKFNWYVDGVEVHNAKTKPREEQYNSTYRVVSVLTVLHQDWLNGKEYKCKVSNKALPAPIEKTISKAKGQPREPQVYTLPPSRDELTKNQVSLTCLVKGFYPSDIAVEWESNGQPENNYKTTPPVLDSDGSFFLYSKLTVDKSRWQQGNVFSCSVMHEALHNHYTQKSLSLSPG

SEQ ID NO: 18 - protein, 447 aa, Artificial Sequence
  T33H / N57H variant of ipilimumab HC
QVQLVESGGGVVQPGRSLRLSCAASGFTFSSYHMHWVRQAPGKGLEWVTFISYDGNHKYYADSVKGRFTISRDNSKNTLYLQMNSLRAEDTAIYYCARTGWLGPFDYWGQGTLVTVSSASTKGPSVFPLAPSSKSTSGGTAALGCLVKDYFPEPVTVSWNSGALTSGVHTFPAVLQSSGLYSLSSVVTVPSSSLGTQTYICNVNHKPSNTKVDKRVEPKSCDKTHTCPPCPAPELLGGPSVFLFPPKPKDTLMISRTPEVTCVVVDVSHEDPEVKFNWYVDGVEVHNAKTKPREEQYNSTYRVVSVLTVLHQDWLNGKEYKCKVSNKALPAPIEKTISKAKGQPREPQVYTLPPSRDELTKNQVSLTCLVKGFYPSDIAVEWESNGQPENNYKTTPPVLDSDGSFFLYSKLTVDKSRWQQGNVFSCSVMHEALHNHYTQKSLSLSPG

SEQ ID NO: 19 - protein, 447 aa, Artificial Sequence
  N56H variant of ipilimumab HC
QVQLVESGGGVVQPGRSLRLSCAASGFTFSSYTMHWVRQAPGKGLEWVTFISYDGHNKYYADSVKGRFTISRDNSKNTLYLQMNSLRAEDTAIYYCARTGWLGPFDYWGQGTLVTVSSASTKGPSVFPLAPSSKSTSGGTAALGCLVKDYFPEPVTVSWNSGALTSGVHTFPAVLQSSGLYSLSSVVTVPSSSLGTQTYICNVNHKPSNTKVDKRVEPKSCDKTHTCPPCPAPELLGGPSVFLFPPKPKDTLMISRTPEVTCVVVDVSHEDPEVKFNWYVDGVEVHNAKTKPREEQYNSTYRVVSVLTVLHQDWLNGKEYKCKVSNKALPAPIEKTISKAKGQPREPQVYTLPPSRDELTKNQVSLTCLVKGFYPSDIAVEWESNGQPENNYKTTPPVLDSDGSFFLYSKLTVDKSRWQQGNVFSCSVMHEALHNHYTQKSLSLSPG

SEQ ID NO: 20 - protein, 447 aa, Artificial Sequence
  S31H / T99H variant of ipilimumab HC
QVQLVESGGGVVQPGRSLRLSCAASGFTFSHYTMHWVRQAPGKGLEWVTFISYDGNNKYYADSVKGRFTISRDNSKNTLYLQMNSLRAEDTAIYYCARHGWLGPFDYWGQGTLVTVSSASTKGPSVFPLAPSSKSTSGGTAALGCLVKDYFPEPVTVSWNSGALTSGVHTFPAVLQSSGLYSLSSVVTVPSSSLGTQTYICNVNHKPSNTKVDKRVEPKSCDKTHTCPPCPAPELLGGPSVFLFPPKPKDTLMISRTPEVTCVVVDVSHEDPEVKFNWYVDGVEVHNAKTKPREEQYNSTYRVVSVLTVLHQDWLNGKEYKCKVSNKALPAPIEKTISKAKGQPREPQVYTLPPSRDELTKNQVSLTCLVKGFYPSDIAVEWESNGQPENNYKTTPPVLDSDGSFFLYSKLTVDKSRWQQGNVFSCSVMHEALHNHYTQKSLSLSPG

SEQ ID NO: 21 - protein, 215 aa, Homo sapiens
EIVLTQSPGTLSLSPGERATLSCRASQSVGSSYLAWYQQKPGQAPRLLIYGAFSRATGIPDRFSGSGSGTDFTLTISRLEPEDFAVYYCQQYGSSPWTFGQGTKVEIKRTVAAPSVFIFPPSDEQLKSGTASVVCLLNNFYPREAKVQWKVDNALQSGNSQESVTEQDSKDSTYSLSSTLTLSKADYEKHKVYACEVTHQGLSSPVTKSFNRGEC

SEQ ID NO: 22 - protein, 215 aa, Artificial Sequence
  S28E / S31D variant of ipilimumab LC
EIVLTQSPGTLSLSPGERATLSCRASQEVGDSYLAWYQQKPGQAPRLLIYGAFSRATGIPDRFSGSGSGTDFTLTISRLEPEDFAVYYCQQYGSSPWTFGQGTKVEIKRTVAAPSVFIFPPSDEQLKSGTASVVCLLNNFYPREAKVQWKVDNALQSGNSQESVTEQDSKDSTYSLSSTLTLSKADYEKHKVYACEVTHQGLSSPVTKSFNRGEC

SEQ ID NO: 23 - protein, 215 aa, Artificial Sequence
  S28E / S31D / Y33E variant of ipilimumab LC
EIVLTQSPGTLSLSPGERATLSCRASQEVGDSELAWYQQKPGQAPRLLIYGAFSRATGIPDRFSGSGSGTDFTLTISRLEPEDFAVYYCQQYGSSPWTFGQGTKVEIKRTVAAPSVFIFPPSDEQLKSGTASVVCLLNNFYPREAKVQWKVDNALQSGNSQESVTEQDSKDSTYSLSSTLTLSKADYEKHKVYACEVTHQGLSSPVTKSFNRGEC

SEQ ID NO: 24 - protein, 215 aa, Artificial Sequence
  S28E variant of ipilimumab LC
EIVLTQSPGTLSLSPGERATLSCRASQEVGSSYLAWYQQKPGQAPRLLIYGAFSRATGIPDRFSGSGSGTDFTLTISRLEPEDFAVYYCQQYGSSPWTFGQGTKVEIKRTVAAPSVFIFPPSDEQLKSGTASVVCLLNNFYPREAKVQWKVDNALQSGNSQESVTEQDSKDSTYSLSSTLTLSKADYEKHKVYACEVTHQGLSSPVTKSFNRGEC

SEQ ID NO: 25 - protein, 215 aa, Artificial Sequence
  S31D variant of ipilimumab LC
EIVLTQSPGTLSLSPGERATLSCRASQSVGDSYLAWYQQKPGQAPRLLIYGAFSRATGIPDRFSGSGSGTDFTLTISRLEPEDFAVYYCQQYGSSPWTFGQGTKVEIKRTVAAPSVFIFPPSDEQLKSGTASVVCLLNNFYPREAKVQWKVDNALQSGNSQESVTEQDSKDSTYSLSSTLTLSKADYEKHKVYACEVTHQGLSSPVTKSFNRGEC

SEQ ID NO: 26 - protein, 215 aa, Artificial Sequence
  Y33E variant of ipilimumab LC
EIVLTQSPGTLSLSPGERATLSCRASQSVGSSELAWYQQKPGQAPRLLIYGAFSRATGIPDRFSGSGSGTDFTLTISRLEPEDFAVYYCQQYGSSPWTFGQGTKVEIKRTVAAPSVFIFPPSDEQLKSGTASVVCLLNNFYPREAKVQWKVDNALQSGNSQESVTEQDSKDSTYSLSSTLTLSKADYEKHKVYACEVTHQGLSSPVTKSFNRGEC

SEQ ID NO: 27 - protein, 215 aa, Artificial Sequence
  S28E / S31E variant of ipilimumab LC
EIVLTQSPGTLSLSPGERATLSCRASQEVGESYLAWYQQKPGQAPRLLIYGAFSRATGIPDRFSGSGSGTDFTLTISRLEPEDFAVYYCQQYGSSPWTFGQGTKVEIKRTVAAPSVFIFPPSDEQLKSGTASVVCLLNNFYPREAKVQWKVDNALQSGNSQESVTEQDSKDSTYSLSSTLTLSKADYEKHKVYACEVTHQGLSSPVTKSFNRGEC

SEQ ID NO: 28 - protein, 215 aa, Artificial Sequence
  S28E / S31E / Y33E variant of ipilimumab LC
EIVLTQSPGTLSLSPGERATLSCRASQEVGESELAWYQQKPGQAPRLLIYGAFSRATGIPDRFSGSGSGTDFTLTISRLEPEDFAVYYCQQYGSSPWTFGQGTKVEIKRTVAAPSVFIFPPSDEQLKSGTASVVCLLNNFYPREAKVQWKVDNALQSGNSQESVTEQDSKDSTYSLSSTLTLSKADYEKHKVYACEVTHQGLSSPVTKSFNRGEC

SEQ ID NO: 29 - protein, 215 aa, Artificial Sequence
  S28D / S31D variant of ipilimumab LC
EIVLTQSPGTLSLSPGERATLSCRASQDVGDSYLAWYQQKPGQAPRLLIYGAFSRATGIPDRFSGSGSGTDFTLTISRLEPEDFAVYYCQQYGSSPWTFGQGTKVEIKRTVAAPSVFIFPPSDEQLKSGTASVVCLLNNFYPREAKVQWKVDNALQSGNSQESVTEQDSKDSTYSLSSTLTLSKADYEKHKVYACEVTHQGLSSPVTKSFNRGEC

SEQ ID NO: 30 - protein, 215 aa, Artificial Sequence
  S28D / S31E variant of ipilimumab LC
EIVLTQSPGTLSLSPGERATLSCRASQDVGESYLAWYQQKPGQAPRLLIYGAFSRATGIPDRFSGSGSGTDFTLTISRLEPEDFAVYYCQQYGSSPWTFGQGTKVEIKRTVAAPSVFIFPPSDEQLKSGTASVVCLLNNFYPREAKVQWKVDNALQSGNSQESVTEQDSKDSTYSLSSTLTLSKADYEKHKVYACEVTHQGLSSPVTKSFNRGEC

SEQ ID NO: 31 - protein, 118 aa, Artificial Sequence
  Ipilimumab (human sequence) with up to three modifications
  MISC_FEATURE (31)..(31): Xaa is S or H
  MISC_FEATURE (56)..(56): Xaa is N or H
  MISC_FEATURE (99)..(99): Xaa is T or H
QVQLVESGGGVVQPGRSLRLSCAASGFTFSXYTMHWVRQAPGKGLEWVTFISYDGXNKYYADSVKGRFTISRDNSKNTLYLQMNSLRAEDTAIYYCARXGWLGPFDYWGQGTLVTVSS

SEQ ID NO: 32 - protein, 108 aa, Artificial Sequence
  Ipilimumab (human sequence) with up to three modifications
  MISC_FEATURE (28)..(28): Xaa is S, D or E
  MISC_FEATURE (31)..(31): Xaa is S, D or E
  MISC_FEATURE (33)..(33): Xaa is Y, D or E
EIVLTQSPGTLSLSPGERATLSCRASQXVGXSXLAWYQQKPGQAPRLLIYGAFSRATGIPDRFSGSGSGTDFTLTISRLEPEDFAVYYCQQYGSSPWTFGQGTKVEIK

SEQ ID NO: 33 - protein, 10 aa, Homo sapiens
GFTFSSYGMH

SEQ ID NO: 34 - protein, 15 aa, Homo sapiens
VIWYDGSNKYYADSV

SEQ ID NO: 35 - protein, 16 aa, Homo sapiens
DPRGATLYYYYYGMDV

SEQ ID NO: 36 - protein, 11 aa, Homo sapiens
RASQSINSYLD

SEQ ID NO: 37 - protein, 7 aa, Homo sapiens
AASSLQS

SEQ ID NO: 38 - protein, 9 aa, Homo sapiens
QQYYSTPFT

SEQ ID NO: 39 - protein, 125 aa, Homo sapiens
QVQLVESGGGVVQPGRSLRLSCAASGFTFSSYGMHWVRQAPGKGLEWVAVIWYDGSNKYYADSVKGRFTISRDNSKNTLYLQMNSLRAEDTAVYYCARDPRGATLYYYYYGMDVWGQGTTVTVSS

SEQ ID NO: 40 - protein, 107 aa, Homo sapiens
DIQMTQSPSSLSASVGDRVTITCRASQSINSYLDWYQQKPGKAPKLLIYAASSLQSGVPSRFSGSGSGTDFTLTISSLQPEDFATYYCQQYYSTPFTFGPGTKVEIK

SEQ ID NO: 41 - protein, 450 aa, Homo sapiens
QVQLVESGGGVVQPGRSLRLSCAASGFTFSSYGMHWVRQAPGKGLEWVAVIWYDGSNKYYADSVKGRFTISRDNSKNTLYLQMNSLRAEDTAVYYCARDPRGATLYYYYYGMDVWGQGTTVTVSSASTKGPSVFPLAPCSRSTSESTAALGCLVKDYFPEPVTVSWNSGALTSGVHTFPAVLQSSGLYSLSSVVTVPSSNFGTQTYTCNVDHKPSNTKVDKTVERKCCVECPPCPAPPVAGPSVFLFPPKPKDTLMISRTPEVTCVVVDVSHEDPEVQFNWYVDGVEVHNAKTKPREEQFNSTFRVVSVLTVVHQDWLNGKEYKCKVSNKGLPAPIEKTISKTKGQPREPQVYTLPPSREEMTKNQVSLTCLVKGFYPSDIAVEWESNGQPENNYKTTPPMLDSDGSFFLYSKLTVDKSRWQQGNVFSCSVMHEALHNHYTQKSLSLSPG

SEQ ID NO: 42 - protein, 214 aa, Homo sapiens
DIQMTQSPSSLSASVGDRVTITCRASQSINSYLDWYQQKPGKAPKLLIYAASSLQSGVPSRFSGSGSGTDFTLTISSLQPEDFATYYCQQYYSTPFTFGPGTKVEIKRTVAAPSVFIFPPSDEQLKSGTASVVCLLNNFYPREAKVQWKVDNALQSGNSQESVTEQDSKDSTYSLSSTLTLSKADYEKHKVYACEVTHQGLSSPVTKSFNRGEC

SEQ ID NO: 43 - protein, 125 aa, Artificial Sequence
  Human sequence with one or more His modifications
  MISC_FEATURE (30)..(30): Xaa is S or H
  MISC_FEATURE (31)..(31): Xaa is S or H
  MISC_FEATURE (52)..(52): Xaa is W or H
  MISC_FEATURE (53)..(53): Xaa is Y or H
  MISC_FEATURE (54)..(54): Xaa is D or H
  MISC_FEATURE (56)..(56): Xaa is S or H
  MISC_FEATURE (57)..(57): Xaa is N or H
  MISC_FEATURE (101)..(101): Xaa is R or H
  MISC_FEATURE (103)..(103): Xaa is A or H
QVQLVESGGGVVQPGRSLRLSCAASGFTFXXYGMHWVRQAPGKGLEWVAVIXXXGXXKYYADSVKGRFTISRDNSKNTLYLQMNSLRAEDTAVYYCARDPXGXTLYYYYYGMDVWGQGTTVTVSS

SEQ ID NO: 44 - protein, 107 aa, Artificial Sequence
  Human sequence with one or more Asp or Glu modifications
  MISC_FEATURE (28)..(28): Xaa is S, D or E
  MISC_FEATURE (30)..(30): Xaa is N, D or E
  MISC_FEATURE (31)..(31): Xaa is S, D or E
  MISC_FEATURE (32)..(32): Xaa is Y, D or E
DIQMTQSPSSLSASVGDRVTITCRASQXIXXXLDWYQQKPGKAPKLLIYAASSLQSGVPSRFSGSGSGTDFTLTISSLQPEDFATYYCQQYYSTPFTFGPGTKVEIK